European Patent Application EP 4 321 538 A1, published February 14, 2024. Title: Fusion protein of antigen-binding molecule and streptavidin mutant. Applicant: Savid Therapeutics Inc. The sequence listing filed with the application follows.

SEQUENCE LISTING (27 sequences)

SEQ ID NO: 1 - protein, 133 aa, Artificial Sequence
  Description of Artificial Sequence: Recombinant protein
AEAGITGTWSDQLGDTFIVTAGADGALTGTYENAVGGAESRYVLTGRYDSAPATDGSGTALGWTVAWKNNSKNAHSATTWSGQYVGGADAKINTQWLLTSGTTNANAWKSTLVGHDTFTKVKPSAASHHHHHH

SEQ ID NO: 2 - protein, 58 aa, Artificial Sequence
  Description of Artificial Sequence: Recombinant protein
VDNKFNKEMRNAYWEIALLPNLNNQQKRAFIRSIYDDPSQSANLLAEAKKLNDAQAPK

SEQ ID NO: 3 - DNA, 636 bp, Artificial Sequence
  Description of Artificial Sequence: Recombinant DNA
  CDS (1)..(636)
atggtggacaacaaattcaacaaagagatgcgcaatgcgtactgggaaattgccctgttaccgaacctgaacaaccagcagaaacgtgccttcattcgcagcatctatgacgatccaagccaatctgcgaatctgcttgcagaagcgaagaaactgaatgatgctcaagctccgaaaagcggaggcggcggcgggtctggtggtggcggtggcagtggcggaggtggcggttcagcggaagccggtattaccgggacctggtccgatcaactcggcgacacgtttatcgtgacagcaggcgcggatggcgcgctgacagggacgtacgagaatgcggtaggcggtgcggaaagccgctatgtgttgaccggtcgttacgattcggctccggctacggatggttccggtacagccttagggtggaccgttgcgtggaagaacaactcgaagaatgcccacagtgctaccacttggtcaggccagtatgttggcggggcggatgcgaaaatcaacactcagtggcttctgaccagcggaaccacgaatgccaatgcgtggaaatccacgctggtcggtcatgacacctttaccaaagtcaaaccgagtgcagcatcgcatcatcaccaccatcattaa

SEQ ID NO: 4 - protein, 211 aa, Artificial Sequence
  Description of Artificial Sequence: Recombinant protein
MVDNKFNKEMRNAYWEIALLPNLNNQQKRAFIRSIYDDPSQSANLLAEAKKLNDAQAPKSGGGGGSGGGGGSGGGGGSAEAGITGTWSDQLGDTFIVTAGADGALTGTYENAVGGAESRYVLTGRYDSAPATDGSGTALGWTVAWKNNSKNAHSATTWSGQYVGGADAKINTQWLLTSGTTNANAWKSTLVGHDTFTKVKPSAASHHHHHH

SEQ ID NO: 5 - DNA, 29 bp, Artificial Sequence
  Description of Artificial Sequence: Synthesized DNA
catggtatatctccttcttaaagttaaac

SEQ ID NO: 6 - DNA, 30 bp, Artificial Sequence
  Description of Artificial Sequence: Synthesized DNA
cgcagcttaattaacctaggctgctgccac

SEQ ID NO: 7 - DNA, 39 bp, Artificial Sequence
  Description of Artificial Sequence: Synthesized DNA
aggagatataccatggtggacaacaaattcaacaaagag

SEQ ID NO: 8 - DNA, 41 bp, Artificial Sequence
  Description of Artificial Sequence: Synthesized DNA
gttaattaagctgcgttaatgatggtggtgatgatgcgatg

SEQ ID NO: 9 - protein, 58 aa, Artificial Sequence [sequence omitted]

SEQ ID NO: 10 - protein, 200 aa, Artificial Sequence
  Description of Artificial Sequence: recombinant protein
MVDNKFNKEMRNAYWEIALLPNLNNQQKRAFIRSIYDDPSQSANLLAEAKKLNDAQAPKSGGGGGSGGGGGSGGGGGSAEAGITGTWSDQLGDTFIVTAGADGALTGTYENAVGGAESRYVLTGRYDSAPATDGSGTALGWTVAWKNNSKNAHSATTWSGQYVGGADAKINTQWLLTSGTTNANAWKSTLVGHDTFTKVK

SEQ ID NO: 11 - DNA, 30 bp, Artificial Sequence
  Description of Artificial Sequence: Synthesized DNA
aagtcaaataacgcagcttaattaacctag

SEQ ID NO: 12 - DNA, 31 bp, Artificial Sequence
  Description of Artificial Sequence: Synthesized DNA
tgcgttatttgactttggtaaaggtgtcatg

SEQ ID NO: 13 - DNA, 603 bp, Artificial Sequence
  Description of Artificial Sequence: Recombinant DNA
atggtggacaacaaattcaacaaagagatgcgcaatgcgtactgggaaattgccctgttaccgaacctgaacaaccagcagaaacgtgccttcattcgcagcatctatgacgatccaagccaatctgcgaatctgcttgcagaagcgaagaaactgaatgatgctcaagctccgaaaagcggaggcggcggcgggtctggtggtggcggtggcagtggcggaggtggcggttcagcggaagccggtattaccgggacctggtccgatcaactcggcgacacgtttatcgtgacagcaggcgcggatggcgcgctgacagggacgtacgagaatgcggtaggcggtgcggaaagccgctatgtgttgaccggtcgttacgattcggctccggctacggatggttccggtacagccttagggtggaccgttgcgtggaagaacaactcgaagaatgcccacagtgctaccacttggtcaggccagtatgttggcggggcggatgcgaaaatcaacactcagtggcttctgaccagcggaaccacgaatgccaatgcgtggaaatccacgctggtcggtcatgacacctttaccaaagtcaaataa

SEQ ID NO: 14 - DNA, 29 bp, Artificial Sequence
  Description of Artificial Sequence: Synthesized DNA
gcggaagccggtattaccgggacctggtc

SEQ ID NO: 15 - DNA, 28 bp, Artificial Sequence
  Description of Artificial Sequence: Synthesized DNA
tttcggagcttgagcatcattcagtttc

SEQ ID NO: 16 - DNA, 72 bp, Artificial Sequence
  Description of Artificial Sequence: Synthesized DNA
gaaactgaatgatgctcaagctccgaaaggaggcggagggtctgcggaagccggtattaccgggacctggtc

SEQ ID NO: 17 - DNA, 72 bp, Artificial Sequence
  Description of Artificial Sequence: Synthesized DNA
gaccaggtcccggtaataccggcttccgcagaccctccgcctcctttcggagcttgagcatcattcagtttc

SEQ ID NO: 18 - DNA, 60 bp, Artificial Sequence
  Description of Artificial Sequence: Synthesized DNA
gctcaagctccgaaaggaggcggagggtctggaggtggcggttcagcggaagccggtatt

SEQ ID NO: 19 - DNA, 60 bp, Artificial Sequence
  Description of Artificial Sequence: Synthesized DNA
aataccggcttccgctgaaccgccacctccagaccctccgcctcctttcggagcttgagc

SEQ ID NO: 20 - DNA, 75 bp, Artificial Sequence
  Description of Artificial Sequence: Synthesized DNA
gctcaagctccgaaaggaggcggagggtctggaggtggcggttcaggtggcggtggcagtgcggaagccggtatt

SEQ ID NO: 21 - DNA, 75 bp, Artificial Sequence
  Description of Artificial Sequence: Synthesized DNA
aataccggcttccgcactgccaccgccacctgaaccgccacctccagaccctccgcctcctttcggagcttgagc

SEQ ID NO: 22 - protein, 186 aa, Artificial Sequence
  Description of Artificial Sequence: recombinant protein
MVDNKFNKEMRNAYWEIALLPNLNNQQKRAFIRSIYDDPSQSANLLAEAKKLNDAQAPKGGGGSAEAGITGTWSDQLGDTFIVTAGADGALTGTYENAVGGAESRYVLTGRYDSAPATDGSGTALGWTVAWKNNSKNAHSATTWSGQYVGGADAKINTQWLLTSGTTNANAWKSTLVGHDTFTKVK

SEQ ID NO: 23 - protein, 191 aa, Artificial Sequence
  Description of Artificial Sequence: recombinant protein
MVDNKFNKEMRNAYWEIALLPNLNNQQKRAFIRSIYDDPSQSANLLAEAKKLNDAQAPKGGGGSGGGGSAEAGITGTWSDQLGDTFIVTAGADGALTGTYENAVGGAESRYVLTGRYDSAPATDGSGTALGWTVAWKNNSKNAHSATTWSGQYVGGADAKINTQWLLTSGTTNANAWKSTLVGHDTFTKVK

SEQ ID NO: 24 - protein, 196 aa, Artificial Sequence
  Description of Artificial Sequence: recombinant protein
MVDNKFNKEMRNAYWEIALLPNLNNQQKRAFIRSIYDDPSQSANLLAEAKKLNDAQAPKGGGGSGGGGSGGGGSAEAGITGTWSDQLGDTFIVTAGADGALTGTYENAVGGAESRYVLTGRYDSAPATDGSGTALGWTVAWKNNSKNAHSATTWSGQYVGGADAKINTQWLLTSGTTNANAWKSTLVGHDTFTKVK

SEQ ID NO: 25 - DNA, 561 bp, Artificial Sequence
  Description of Artificial Sequence: Recombinant DNA
atggtggacaacaaattcaacaaagagatgcgcaatgcgtactgggaaattgccctgttaccgaacctgaacaaccagcagaaacgtgccttcattcgcagcatctatgacgatccaagccaatctgcgaatctgcttgcagaagcgaagaaactgaatgatgctcaagctccgaaaggaggcggagggtctgcggaagccggtattaccgggacctggtccgatcaactcggcgacacgtttatcgtgacagcaggcgcggatggcgcgctgacagggacgtacgagaatgcggtaggcggtgcggaaagccgctatgtgttgaccggtcgttacgattcggctccggctacggatggttccggtacagccttagggtggaccgttgcgtggaagaacaactcgaagaatgcccacagtgctaccacttggtcaggccagtatgttggcggggcggatgcgaaaatcaacactcagtggcttctgaccagcggaaccacgaatgccaatgcgtggaaatccacgctggtcggtcatgacacctttaccaaagtcaaataa

SEQ ID NO: 26 - DNA, 576 bp, Artificial Sequence
  Description of Artificial Sequence: Recombinant DNA
atggtggacaacaaattcaacaaagagatgcgcaatgcgtactgggaaattgccctgttaccgaacctgaacaaccagcagaaacgtgccttcattcgcagcatctatgacgatccaagccaatctgcgaatctgcttgcagaagcgaagaaactgaatgatgctcaagctccgaaaggaggcggagggtctggaggtggcggttcagcggaagccggtattaccgggacctggtccgatcaactcggcgacacgtttatcgtgacagcaggcgcggatggcgcgctgacagggacgtacgagaatgcggtaggcggtgcggaaagccgctatgtgttgaccggtcgttacgattcggctccggctacggatggttccggtacagccttagggtggaccgttgcgtggaagaacaactcgaagaatgcccacagtgctaccacttggtcaggccagtatgttggcggggcggatgcgaaaatcaacactcagtggcttctgaccagcggaaccacgaatgccaatgcgtggaaatccacgctggtcggtcatgacacctttaccaaagtcaaataa

SEQ ID NO: 27 - DNA, 591 bp, Artificial Sequence
  Description of Artificial Sequence: Recombinant DNA
atggtggacaacaaattcaacaaagagatgcgcaatgcgtactgggaaattgccctgttaccgaacctgaacaaccagcagaaacgtgccttcattcgcagcatctatgacgatccaagccaatctgcgaatctgcttgcagaagcgaagaaactgaatgatgctcaagctccgaaaggaggcggagggtctggaggtggcggttcaggtggcggtggcagtgcggaagccggtattaccgggacctggtccgatcaactcggcgacacgtttatcgtgacagcaggcgcggatggcgcgctgacagggacgtacgagaatgcggtaggcggtgcggaaagccgctatgtgttgaccggtcgttacgattcggctccggctacggatggttccggtacagccttagggtggaccgttgcgtggaagaacaactcgaagaatgcccacagtgctaccacttggtcaggccagtatgttggcggggcggatgcgaaaatcaacactcagtggcttctgaccagcggaaccacgaatgccaatgcgtggaaatccacgctggtcggtcatgacacctttaccaaagtcaaataa